European Patent Specification EP 3 914 293 B1, published July 3, 2024. Title: VACCINATION AGAINST CORONAVIRUS WITH POLIOMYELITIS VACCINE. Applicant: Xie, Qiyi. The sequence listing filed with the application follows.

SEQUENCE LISTING (4 sequences)

SEQ ID NO: 1 - protein, 430 aa, Homo sapiens
EGSKEPAVLNPKDPRLKTDFEEAIFSKYTGNKIMLMDEYMEEAVDHYVGCLEPLDISVDPIPLESAMYGMDGLEALDLTTSAGFPYLLQGKKKRDIFNRHTRDTTEMTKMLEKYGVDLPFVTFVKDELRSREKVEKGKSRLIEASSLNDSVAMRVAFGNLYATFHSNPGTATGSAVGCDPDIFWSKIPILLDGEIFAFDYTGYDASLSPVWFACLKKVLIKLGYTHQTSFIDYLCHSVHLYKDRKYIVNGGMPSGSSGTSIFNTMINNIIIRTLLIRVYKGIDLDQFKMIAYGDDVIASYPHKIDPGLLAEAGKHYGLVMTPADKGTSFVDTNWENVTFLKRYFRADDQYPFLIHPVMPMKEIHESIRWTKDPRNTQDHVRSLCYLAWHNGEEAYDEFCRKIRSVPVGRALTLPAYSSLRRKWLDSFLER

SEQ ID NO: 2 - protein, 932 aa, Homo sapiens
SADAQSFLNRVCGVSAARLTPCGTGTSTDVVYRAFDIYNDKVAGFAKFLKTNCCRFQEKDEDDNLIDSYFVVKRHTFSNYQHEETIYNLLKDCPAVAKHDFFKFRIDGDMVPHISRQRLTKYTMADLVYALRHFDEGNCDTLKEILVTYNCCDDDYFNKKDWYDFVENPDILRVYANLGERVRQALLKTVQFCDAMRNAGIVGVLTLDNQDLNGNWYDFGDFIQTTPGSGVPVVDSYYSLLMPILTLTRALTAESHVDTDLTKPYIKWDLLKYDFTEERLKLFDRYFKYWDQTYHPNCVNCLDDRCILHCANFNVLFSTVFPPTSFGPLVRKIFVDGVPFVVSTGYHFRELGVVHNQDVNLHSSRLSFKELLVYAADPAMHAASGNLLLDKRTTCFSVAALTNNVAFQTVKPGNFNKDFYDFAVSKGFFKEGSSVELKHFFFAQDGNAAISDYDYYRYNLPTMCDIRQLLFVVEVVDKYFDCYDGGCINANQVIVNNLDKSAGFPFNKWGKARLYYDSMSYEDQDALFAYTKRNVIPTITQMNLKYAISAKNRARTVAGVSICSTMTNRQFHQKLLKSIAATRGATVVIGTSKFYGGWHNMLKTVYSDVENPHLMGWDYPKCDRAMPNMLRIMASLVLARKHTTCCSLSHRFYRLANECAQVLSEMVMCGGSLYVKPGGTSSGDATTAYANSVFNICQAVTANVNALLSTDGNKIADKYVRNLQHRLYECLYRNRDVDTDFVNEFYAYLRKHFSMMILSDDAVVCFNSTYASQGLVASIKNFKSVLYYQNNVFMSEAKCWTETDLTKGPHEFCSQHTMLVKQGDDYVYLPYPDPSRILGAGCFVDDIVKTDGTLMIERFVSLAIDAYPLTKHPNQEYADVFHLYLQYIRKLHDELTGHMLDMYSVMLTNDNTSRYWEPEFYEAMYTPHTVLQ

SEQ ID NO: 3 - protein, 331 aa, Homo sapiens
SADAQSFLNRVCGVSAARLTPCGTGTSTDVVYRAFDIYNDKVAGFAKFLKTNCCRFQEKDEDDNLIDSYFVVKRHTFSNYQHEETIYNLLKDCPAVAKHDFFKFRIDGDMVPHISRQRLTKYTMADLVYALRHFDEGNCDTLKEILVTYNCCDDDYFNKKDWYDFVENPDILRVYANLGERVRQALLKTVQFCDAMRNAGIVGVLTLDNQDLNGNWYDFGDFIQTTPGSGVPVVDSYYSLLMPILTLTRALTAESHVDTDLTKPYIKWDLLKYDFTEERLKLFDRYFKYWDQTYHPNCVNCLDDRCILHCANFNVLFSTVFPPTSFGPLVR

SEQ ID NO: 4 - protein, 601 aa, Homo sapiens
KIFVDGVPFVVSTGYHFRELGVVHNQDVNLHSSRLSFKELLVYAADPAMHAASGNLLLDKRTTCFSVAALTNNVAFQTVKPGNFNKDFYDFAVSKGFFKEGSSVELKHFFFAQDGNAAISDYDYYRYNLPTMCDIRQLLFVVEVVDKYFDCYDGGCINANQVIVNNLDKSAGFPFNKWGKARLYYDSMSYEDQDALFAYTKRNVIPTITQMNLKYAISAKNRARTVAGVSICSTMTNRQFHQKLLKSIAATRGATVVIGTSKFYGGWHNMLKTVYSDVENPHLMGWDYPKCDRAMPNMLRIMASLVLARKHTTCCSLSHRFYRLANECAQVLSEMVMCGGSLYVKPGGTSSGDATTAYANSVFNICQAVTANVNALLSTDGNKIADKYVRNLQHRLYECLYRNRDVDTDFVNEFYAYLRKHFSMMILSDDAVVCFNSTYASQGLVASIKNFKSVLYYQNNVFMSEAKCWTETDLTKGPHEFCSQHTMLVKQGDDYVYLPYPDPSRILGAGCFVDDIVKTDGTLMIERFVSLAIDAYPLTKHPNQEYADVFHLYLQYIRKLHDELTGHMLDMYSVMLTNDNTSRYWEPEFYEAMYTPHTVLQ